European Patent Specification EP 3 592 379 B1, published April 24, 2024. Title: Universal anti-CD22 CHIMERIC ANTIGEN RECEPTOR ENGINEERED IMMUNE CELLS. Applicant: Cellectis SA. The sequence listing filed with the application follows.

SEQUENCE LISTING (26 sequences)

SEQ ID NO: 1 - protein, 21 aa, homo sapiens
  CD8alpha signal peptide
MALPVTALLLPLALLLHAARP

SEQ ID NO: 2 - protein, 20 aa, homo sapiens
  signal peptide
METDTLLLWVLLLWVPGSTG

SEQ ID NO: 3 - protein, 16 aa, homo sapiens
  FcgRIIIa hinge
GLAVSTISSFFPPGYQ

SEQ ID NO: 4 - protein, 45 aa, homo sapiens
  CD8alpha hinge
TTTPAPRPPTPAPTIASQPLSLRPEACRPAAGGAVHTRGLDFACD

SEQ ID NO: 5 - protein, 231 aa, homo sapiens
  IgG1 hinge
EPKSPDKTHTCPPCPAPPVAGPSVFLFPPKPKDTLMIARTPEVTCVVVDVSHEDPEVKFNWYVDGVEVHNAKTKPREEQYNSTYRVVSVLTVLHQDWLNGKEYKCKVSNKALPAPIEKTISKAKGQPREPQVYTLPPSRDELTKNQVSLTCLVKGFYPSDIAVEWESNGQPENNYKTTPPVLDSDGSFFLYSKLTVDKSRWQQGNVFSCSVMHEALHNHYTQKSLSLSPGK

SEQ ID NO: 6 - protein, 24 aa, homo sapiens
  CD8alpha transmembrane domain
IYIWAPLAGTCGVLLLSLVITLYC

SEQ ID NO: 7 - protein, 27 aa, homo sapiens
  41BB transmembrane domain
IISFFLALTSTALLFLLFFLTLRFSVV

SEQ ID NO: 8 - protein, 42 aa, homo sapiens
  Fragment of 4-1BB (residues 214-255)
KRGRKKLLYIFKQPFMRPVQTTQEEDGCSCRFPEEEEGGCEL

SEQ ID NO: 9 - protein, 112 aa, homo sapiens
  fragment of T-cell surface glycoprotein CD3 zeta chain
RVKFSRSADAPAYQQGQNQLYNELNLGRREEYDVLDKRRGRDPEMGGKPRRKNPQEGLYNELQKDKMAEAYSEIGMKGERRRGKGHDGLYQGLSTATKDTYDALHMQALPPR

SEQ ID NO: 10 - protein, 15 aa, artificial sequence
  G4Sx3 linker sequence
GGGGSGGGGSGGGGS

SEQ ID NO: 11 - DNA, 1532 bp, homo sapiens
  UCART22
tgatcctcttgtcccacagatatccagaaccctgaccctgccgtgtaccagctgagagaatggctctgcccgtcaccgctctgctgctgccactggccctgctgctgcacgcagcaagaccacaggtgcagctgcagcagagcggccctggcctggtgaagccaagccagacactgtccctgacctgcgccatcagcggcgattccgtgagctccaactccgccgcctggaattggatcaggcagtccccttctcggggcctggagtggctgggaaggacatactatcggtctaagtggtacaacgattatgccgtgtctgtgaagagcagaatcacaatcaaccctgacacctccaagaatcagttctctctgcagctgaatagcgtgacaccagaggacaccgccgtgtactattgcgccagggaggtgaccggcgacctggaggatgcctttgacatctggggccagggcacaatggtgaccgtgtctagcggaggaggaggatccggaggaggaggatctggcggcggcggcagcgatatccagatgacacagtccccatcctctctgagcgcctccgtgggcgacagagtgacaatcacctgtagggcctcccagaccatctggtcttacctgaactggtatcagcagaggcccggcaaggcccctaatctgctgatctacgcagcaagctccctgcagagcggagtgccatccagattctctggcaggggctccggcacagacttcaccctgaccatctctagcctgcaggccgaggacttcgccacctactattgccagcagtcttatagcatcccccagacatttggccagggcaccaagctggagatcaagaccacaaccccagcaccaaggccacctacacctgcaccaaccatcgcctctcagcccctgagcctgagacctgaggcatgtaggccagcagcaggaggagcagtccatacaaggggtctggattttgcatgcgacatctacatctgggcacctctggcaggaacatgtggcgtgctcctgctcagcctggtcatcaccctgtactgcaagagaggcaggaagaagctgctgtatatcttcaagcagcccttcatgcgccccgtgcagacaacccaggaggaggatggctgctcctgtaggttcccagaagaggaggagggaggatgtgagctgcgcgtgaagttttcccggtctgccgacgcacctgcataccagcagggccagaaccagctgtataacgagctgaatctgggccggagagaggagtacgatgtgctggacaagaggcgcggcagagatccagagatgggcggcaagccccggagaaagaaccctcaggagggcctgtacaatgagctgcagaaggataagatggccgaggcctattctgagatcggcatgaagggagagaggcgccggggcaagggacacgacggactgtaccagggactgagcacagccaccaaggatacctatgacgccctgcatatgcaggcactgcctccaaggtga

SEQ ID NO: 12 - protein, 124 aa, artificial sequence
  971- heavy chain
QVQLQQSGPGLVKPSQTLSLTCAISGDSVSSNSAAWNWIRQSPSRGLEWLGRTYYRSKWYNDYAVSVKSRITINPDTSKNQFSLQLNSVTPEDTAVYYCAREVTGDLEDAFDIWGQGTMVTVSS

SEQ ID NO: 13 - protein, 107 aa, artificial sequence
  971- light chain
DIQMTQSPSSLSASVGDRVTITCRASQTIWSYLNWYQQRPGKAPNLLIYAASSLQSGVPSRFSGRGSGTDFTLTISSLQAEDFATYYCQQSYSIPQTFGQGTKLEIK

SEQ ID NO: 14 - protein, 461 aa, artificial sequence
  971-v1 polypeptide CAR sequence
MALPVTALLLPLALLLHAARPQVQLQQSGPGLVKPSQTLSLTCAISGDSVSSNSAAWNWIRQSPSRGLEWLGRTYYRSKWYNDYAVSVKSRITINPDTSKNQFSLQLNSVTPEDTAVYYCAREVTGDLEDAFDIWGQGTMVTVSSGGGGSGGGGSGGGGSDIQMTQSPSSLSASVGDRVTITCRASQTIWSYLNWYQQRPGKAPNLLIYAASSLQSGVPSRFSGRGSGTDFTLTISSLQAEDFATYYCQQSYSIPQTFGQGTKLEIKGLAVSTISSFFPPGYQIYIWAPLAGTCGVLLLSLVITLYCKRGRKKLLYIFKQPFMRPVQTTQEEDGCSCRFPEEEEGGCELRVKFSRSADAPAYQQGQNQLYNELNLGRREEYDVLDKRRGRDPEMGGKPRRKNPQEGLYNELQKDKMAEAYSEIGMKGERRRGKGHDGLYQGLSTATKDTYDALHMQALPPR

SEQ ID NO: 15 - protein, 490 aa, artificial sequence
  971-v3 polypeptide CAR sequence
MALPVTALLLPLALLLHAARPQVQLQQSGPGLVKPSQTLSLTCAISGDSVSSNSAAWNWIRQSPSRGLEWLGRTYYRSKWYNDYAVSVKSRITINPDTSKNQFSLQLNSVTPEDTAVYYCAREVTGDLEDAFDIWGQGTMVTVSSGGGGSGGGGSGGGGSDIQMTQSPSSLSASVGDRVTITCRASQTIWSYLNWYQQRPGKAPNLLIYAASSLQSGVPSRFSGRGSGTDFTLTISSLQAEDFATYYCQQSYSIPQTFGQGTKLEIKTTTPAPRPPTPAPTIASQPLSLRPEACRPAAGGAVHTRGLDFACDIYIWAPLAGTCGVLLLSLVITLYCKRGRKKLLYIFKQPFMRPVQTTQEEDGCSCRFPEEEEGGCELRVKFSRSADAPAYQQGQNQLYNELNLGRREEYDVLDKRRGRDPEMGGKPRRKNPQEGLYNELQKDKMAEAYSEIGMKGERRRGKGHDGLYQGLSTATKDTYDALHMQALPPR

SEQ ID NO: 16 - protein, 530 aa, artificial sequence
  TAL binding domain  TRAC_T01-L
LTPQQVVAIASNGGGKQALETVQRLLPVLCQAHGLTPQQVVAIASNNGGKQALETVQRLLPVLCQAHGLTPQQVVAIASNGGGKQALETVQRLLPVLCQAHGLTPEQVVAIASHDGGKQALETVQRLLPVLCQAHGLTPEQVVAIASHDGGKQALETVQRLLPVLCQAHGLTPEQVVAIASHDGGKQALETVQRLLPVLCQAHGLTPEQVVAIASNIGGKQALETVQALLPVLCQAHGLTPEQVVAIASHDGGKQALETVQRLLPVLCQAHGLTPEQVVAIASNIGGKQALETVQALLPVLCQAHGLTPQQVVAIASNNGGKQALETVQRLLPVLCQAHGLTPEQVVAIASNIGGKQALETVQALLPVLCQAHGLTPQQVVAIASNGGGKQALETVQRLLPVLCQAHGLTPEQVVAIASNIGGKQALETVQALLPVLCQAHGLTPQQVVAIASNGGGKQALETVQRLLPVLCQAHGLTPEQVVAIASHDGGKQALETVQRLLPVLCQAHGLTPQQVVAIASNGGGRPALE

SEQ ID NO: 17 - protein, 530 aa, artificial sequence
  TAL binding domain TRAC_T01-R
LTPEQVVAIASHDGGKQALETVQRLLPVLCQAHGLTPQQVVAIASNGGGKQALETVQRLLPVLCQAHGLTPEQVVAIASHDGGKQALETVQRLLPVLCQAHGLTPEQVVAIASNIGGKQALETVQALLPVLCQAHGLTPQQVVAIASNNGGKQALETVQRLLPVLCQAHGLTPEQVVAIASHDGGKQALETVQRLLPVLCQAHGLTPQQVVAIASNGGGKQALETVQRLLPVLCQAHGLTPQQVVAIASNNGGKQALETVQRLLPVLCQAHGLTPQQVVAIASNNGGKQALETVQRLLPVLCQAHGLTPQQVVAIASNGGGKQALETVQRLLPVLCQAHGLTPEQVVAIASNIGGKQALETVQALLPVLCQAHGLTPEQVVAIASHDGGKQALETVQRLLPVLCQAHGLTPEQVVAIASNIGGKQALETVQALLPVLCQAHGLTPEQVVAIASHDGGKQALETVQRLLPVLCQAHGLTPQQVVAIASNNGGKQALETVQRLLPVLCQAHGLTPQQVVAIASNGGGRPALE

SEQ ID NO: 18 - DNA, 49 bp, artificial sequence
  target TALEN TRAC_T01
ttgtcccacagatatccagaaccctgaccctgccgtgtaccagctgaga

SEQ ID NO: 19 - protein, 9 aa, artificial sequence
  Mimotope of CD20 antigen
CPYSNPSLC

SEQ ID NO: 20 - DNA, 1473 bp, artificial sequence
  CAR 11 dis 16
atggctctgcccgtcaccgctctgctgctgccactggccctgctgctgcacgcagcaagaccacaggtgcagctgcagcagagcggccctggcctggtgaagccaagccagacactgtccctgacctgcgccatcagcggcgattccgtgagctccaactccgccgcctggaattggatcaggcagtccccttctcggggcctggagtggctgggaaggacatactatcggtctaagtggtacaacgattatgccgtgtctgtgaagagcagaatcacaatcaaccctgacacctccaagaatcagttctctctgcagctgaatagcgtgacaccagaggacaccgccgtgtactattgcgccagggaggtgaccggcgacctggaggatgcctttgacatctggggccagggcacaatggtgaccgtgtctagcggaggaggaggatccggaggaggaggatctggcggcggcggcagcgatatccagatgacacagtccccatcctctctgagcgcctccgtgggcgacagagtgacaatcacctgtagggcctcccagaccatctggtcttacctgaactggtatcagcagaggcccggcaaggcccctaatctgctgatctacgcagcaagctccctgcagagcggagtgccatccagattctctggcaggggctccggcacagacttcaccctgaccatctctagcctgcaggccgaggacttcgccacctactattgccagcagtcttatagcatcccccagacatttggccagggcaccaagctggagatcaagaccacaaccccagcaccaaggccacctacacctgcaccaaccatcgcctctcagcccctgagcctgagacctgaggcatgtaggccagcagcaggaggagcagtccatacaaggggtctggattttgcatgcgacatctacatctgggcacctctggcaggaacatgtggcgtgctcctgctcagcctggtcatcaccctgtactgcaagagaggcaggaagaagctgctgtatatcttcaagcagcccttcatgcgccccgtgcagacaacccaggaggaggatggctgctcctgtaggttcccagaagaggaggagggaggatgtgagctgcgcgtgaagttttcccggtctgccgacgcacctgcataccagcagggccagaaccagctgtataacgagctgaatctgggccggagagaggagtacgatgtgctggacaagaggcgcggcagagatccagagatgggcggcaagccccggagaaagaaccctcaggagggcctgtacaatgagctgcagaaggataagatggccgaggcctattctgagatcggcatgaagggagagaggcgccggggcaagggacacgacggactgtaccagggactgagcacagccaccaaggatacctatgacgccctgcatatgcaggcactgcctccaaggtga

SEQ ID NO: 21 - DNA, 59 bp, artificial sequence
  TARGET TALEN(R)
tgatcctcttgtcccacagatatccagaaccctgaccctgccgtgtaccagctgagaga

SEQ ID NO: 22 - DNA, 1473 bp, Artificial sequence; identical to SEQ ID NO: 20
  971-v3 polynucleotide CAR sequence

SEQ ID NO: 23 - protein, 489 aa, artificial sequence
  CAR distal CD22
MALPVTALLLPLALLLHAARPEVQLVESGGGLVKPGGSLKLSCAASGFAFSIYDMSWVRQTPEKRLEWVAYISSGGGTYYPDTVKGRFTISRDNAKNTLYLQMSSLKSEDTAMYYCARHSGYGTHWGVLFAYWGQGTLVTVSAGGGGSGGGGSGGGGSDIQMTQTTSSLSASLGDRVTISCRASQDISNYLNWYQQKPDGTVKLLIYYTSILHSGVPSRFSGSGSGTDYSLTISNLEQEDFATYFCQQGNTLPWTFGGGTKLEIKATTTPAPRPPTPAPTIASQPLSLRPEACRPAAGGAVHTRGLDFACDIYIWAPLAGTCGVLLLSLVITLYCKRGRKKLLYIFKQPFMRPVQTTQEEDGCSCRFPEEEEGGCELRVKFSRSADAPAYQQGQNQLYNELNLGRREEYDVLDKRRGRDPEMGGKPRRKNPQEGLYNELQKDKMAEAYSEIGMKGERRRGKGHDGLYQGLSTATKDTYDALHMQALPPR

SEQ ID NO: 24 - DNA, 1470 bp, artificial sequence
  CAR distal CD22
atggctctgcccgtcaccgctctgctgctgccactggccctgctgctgcacgcagcaaggcctgaggtgcagctggtggaatccggaggaggcctggtgaagcctggcggctctctgaagctgagctgtgccgcctccggcttcgccttttccatctacgacatgtcttgggtgaggcagaccccagagaagcgcctggagtgggtggcctatatcagctccggcggcggcacctactatcccgacacagtgaagggccggttcaccatctctagagataacgccaagaatacactgtacctgcagatgtctagcctgaagagcgaggataccgccatgtactattgcgcaaggcactccggatacggaacacactggggcgtgctgtttgcctattggggccagggcaccctggtgacagtgagcgccggaggaggaggaagcggcggaggaggctccggcggcggcggctctgacatccagatgacccagaccacatcctctctgagcgcctccctgggcgacagggtgacaatctcttgtagagccagccaggatatctccaactacctgaattggtatcagcagaagcctgatggcaccgtgaagctgctgatctactatacatctatcctgcacagcggagtgccatcccggttctctggaagcggatccggaaccgactactctctgacaatcagcaacctggagcaggaggatttcgccacctatttttgccagcagggcaataccctgccttggacatttggcggcggcacaaagctggagatcaaggccaccacaacccctgcaccaaggccaccaacaccagcacctaccatcgcatctcagcctctgagcctgagaccagaggcatgtaggccagcagcaggaggagcagtgcacacaaggggactggattttgcctgtgatatctacatctgggcacctctggcaggaacatgtggcgtgctcctgctcagcctggtcatcaccctgtactgcaagagaggcaggaagaagctgctgtatatcttcaagcagcccttcatgagacccgtgcagacaacccaggaggaggacggctgctcctgtaggttcccagaagaggaggagggaggatgtgagctgcgcgtgaagttttcccggtctgccgatgcacctgcataccagcagggacagaatcagctgtataacgagctgaatctgggccggagagaggagtacgacgtgctggataagaggaggggaagggacccagagatgggaggcaagcctcggagaaagaacccacaggagggcctgtacaatgagctgcagaaggacaagatggccgaggcctattctgagatcggcatgaagggagagaggcgccggggcaagggacacgatggcctgtaccagggcctgtccacagccaccaaggacacctatgatgccctgcatatgcaggcactgcctccaaggtga

SEQ ID NO: 25 - protein, 495 aa, artificial sequence
  description of artificial sequence: synthetic polypeptide
  4G7-CAR version 1
MALPVTALLLPLALLLHAARPEVQLQQSGPELIKPGASVKMSCKASGYTFTSYVMHWVKQKPGQGLEWIGYINPYNDGTKYNEKFKGKATLTSDKSSSTAYMELSSLTSEDSAVYYCARGTYYYGSRVFDYWGQGTTLTVSSGGGGSGGGGSGGGGSDIVMTQAAPSIPVTPGESVSISCRSSKSLLNSNGNTYLYWFLQRPGQSPQLLIYRMSNLASGVPDRFSGSGSGTAFTLRISRVEAEDVGVYYCMQHLEYPFTFGAGTKLELKRADTTTPAPRPPTPAPTIASQPLSLRPEACRPAAGGAVHTRGLDFACDIYIWAPLAGTCGVLLLSLVITLYCKRGRKKLLYIFKQPFMRPVQTTQEEDGCSCRFPEEEEGGCELRVKFSRSADAPAYQQGQNQLYNELNLGRREEYDVLDKRRGRDPEMGGKPRRKNPQEGLYNELQKDKMAEAYSEIGMKGERRRGKGHDGLYQGLSTATKDTYDALHMQALPPR

SEQ ID NO: 26 - protein, 495 aa, artificial sequence
  description of artificial sequence: synthetic polypeptide
  4G7-CAR version 2
METDTLLLWVLLLWVPGSTGEVQLQQSGPELIKPGASVKMSCKASGYTFTSYVMHWVKQKPGQGLEWIGYINPYNDGTKYNEKFKGKATLTSDKSSSTAYMELSSLTSEDSAVYYCARGTYYYGSRVFDYWGQGTTLTVSSGGGGSGGGGSGGGGSDIVMTQAAPSIPVTPGESVSISCRSSKSLLNSNGNTYLYWFLQRPGQSPQLLIYRMSNLASGVPDRFSGSGSGTAFTLRISRVEAEDVGVYYCMQHLEYPFTFGAGTKLELKRSDPTTTPAPRPPTPAPTIASQPLSLRPEACRPAAGGAVHTRGLDFACDIYIWAPLAGTCGVLLLSLVITLYCKRGRKKLLYIFKQPFMRPVQTTQEEDGCSCRFPEEEEGGCELRVKFSRSADAPAYQQGQNQLYNELNLGRREEYDVLDKRRGRDPEMGGKPRRKNPQEGLYNELQKDKMAEAYSEIGMKGERRRGKGHDGLYQGLSTATKDTYDALHMQALPPR